European Patent Specification EP 3 720 466 B1, published September 23, 2026. Title: Treatment of Muscular Dystrophies. Applicant: Royal Holloway and Bedford New College. The sequence listing filed with the application follows.

SEQUENCE LISTING (3 sequences)

SEQ ID NO: 1 - DNA, 11061 bp, Artificial sequence
  Codon optimised dystrophin cDNA
atgctgtggtgggaggaagtggaagattgctacgagcgcgaggacgtgcagaagaaaaccttcaccaaatgggtcaacgcccagttcagcaagttcggcaagcagcacatcgagaacctgttcagcgacctgcaggacggcagaaggctgctggacctgctggaaggcctgaccggccagaagctgcccaaagagaagggcagcaccagagtgcacgccctgaacaacgtgaacaaggccctgagagtgctgcagaacaacaacgtggacctggtcaacatcggcagcaccgacatcgtggacggcaaccacaagctgaccctgggcctgatctggaacatcatcctgcactggcaggtcaaaaacgtgatgaagaacatcatggccggcctgcagcagaccaacagcgagaagatcctgctgagctgggtccgccagagcaccagaaactacccccaggtcaacgtgatcaacttcaccacctcttggagcgacggcctggccctgaacgccctgatccacagccacagacccgacctgttcgactggaacagcgtggtctgccagcagagcgccacccagagactggaacacgccttcaatatcgccagataccagctgggcatcgagaagctgctggatcccgaggacgtggacaccacctaccccgacaagaaatccatcctgatgtacatcaccagcctgttccaggtgctgccccagcaggtctccatcgaggccatccaggaagtggaaatgctgcccagaccccccaaagtgaccaaagaggaacacttccagctgcaccaccagatgcactacagccagcagatcaccgtgtccctggctcagggctacgagagaaccagcagccccaagcccagattcaagagctacgcctacacccaggccgcctacgtgaccaccagcgaccccaccagaagcccattccccagccagcacctggaagcccccgaggacaagagcttcggcagcagcctgatggaaagcgaagtgaacctggacagataccagaccgccctggaagaggtgctgtcctggctgctgtccgccgaggacacactgcaggcccagggcgagatcagcaacgacgtggaagtggtcaaagaccagttccacacccacgagggctacatgatggacctgaccgcccaccagggcagagtgggcaacatcctgcagctgggcagcaagctgatcggcaccggcaagctgagcgaggacgaagagacagaggtgcaggaacagatgaacctgctgaacagcagatgggagtgcctgagagtggccagcatggaaaagcagagcaacctgcacagagtgctgatggatctgcagaaccagaagctgaaagagctgaacgactggctgaccaagaccgaggaacggaccagaaagatggaagaggaacccctgggccccgacctggaagatctgaagagacaggtgcagcagcacaaggtgctgcaggaagatctggaacaggaacaggtccgcgtcaacagcctgacccacatggtggtggtggtggacgagagcagcggcgatcacgccaccgccgctctggaagaacagctgaaggtgctgggcgacagatgggccaacatctgccggtggaccgaggacagatgggtgctgctgcaggacatcctgctgaagtggcagagactgacagaggaacagtgcctgttctccgcctggctgagcgagaaagaggacgccgtcaacaagatccacaccaccggcttcaaggaccagaacgagatgctgagcagcctgcagaaactggccgtgctgaaggccgatctggaaaagaaaaagcagtccatgggcaagctgtacagcctgaagcaggacctgctgtccaccctgaagaacaagagcgtgacccagaaaaccgaggcctggctggacaacttcgccagatgctgggacaacctggtgcagaagctggaaaagagcaccgcccagatcagccaggccgtgaccacaacccagccctccctgacccagaccaccgtgatggaaaccgtgaccactgtgaccacccgcgagcagatcctggtcaaacacgcccaggaagaactgccccctccacccccccagaagaaaagacagatcacagtggacagcgagatcagaaagcggctggatgtggacatcaccgagctgcacagctggatcaccagatccgaggccgtgctgcagagccccgagttcgccatcttcagaaaagagggcaacttctccgacctgaaagaaaaagtgaacgccatcgagagagagaaggccgagaagttcagaaagctgcaggacgccagccgctctgctcaggctctggtggaacagatggtcaacgagggcgtgaacgccgacagcatcaagcaggccagcgagcagctgaactccagatggatcgagttctgccagctgctgtccgagagactgaactggctggaataccagaacaacatcattgccttctacaaccagctccagcagctggaacagatgaccaccaccgccgagaactggctgaagatccagcccaccacccccagcgagcccaccgccatcaagagccagctgaagatctgcaaggacgaagtgaacagactgtctggcctgcagccccagatcgagaggctgaagattcagtctatcgccctgaaagagaaaggccagggccccatgttcctggacgccgacttcgtggccttcaccaaccacttcaaacaggtgttctccgacgtgcaggccagagagaaagagctgcagaccatcttcgacaccctgccccccatgagataccaggaaaccatgagcgccatcagaacctgggtgcagcagagcgagacaaagctgagcatcccccagctgagcgtgaccgactacgagatcatggaacagagactgggcgagctgcaggctctgcagtccagtctgcaggaacagcagagcggcctgtactacctgagcaccaccgtgaaagagatgagcaagaaggccccctccgagatctccagaaagtaccagagcgagttcgaagagatcgagggcagatggaagaagctgtcctctcagctggtggaacactgccagaaactggaagaacagatgaacaagctgcggaagatccagaaccacatccagaccctgaaaaagtggatggccgaggtggacgtgttcctgaaagaggaatggcctgccctgggcgactccgagatcctgaaaaagcagctgaagcagtgcagactgctggtgtccgacatccagacaatccagcccagcctgaactccgtgaatgagggcggccagaagatcaagaacgaggccgagcctgagttcgccagcagactggaaaccgagctgaaagaactgaatacccagtgggaccacatgtgtcagcaggtctacgcccggaaagaggccctgaagggcggcctggaaaagaccgtgtctctgcagaaagacctgtccgagatgcacgagtggatgacccaggccgaggaagagtacctggaaagagacttcgagtacaagacccccgacgagctgcagaaagctgtggaagaaatgaagagggccaaagaagaggcccagcagaaagaggccaaagtcaagctgctgaccgagtccgtgaacagcgtgatcgcccaggcccctcccgtggctcaggaagccctgaagaaagaactggaaacactgaccaccaactaccagtggctgtgcaccagactgaacggcaagtgcaagaccctggaagaagtgtgggcctgctggcacgagctgctgagctacctggaaaaggccaacaagtggctgaacgaggtggaattcaagctgaaaaccaccgagaacatccctggcggcgctgaagagatcagcgaggtgctggacagcctggaaaacctgatgagacacagcgaggacaaccccaaccagatcagaatcctggcccagacactgaccgacggcggcgtgatggacgagctgatcaacgaggaactggaaaccttcaacagccggtggcgcgagctgcacgaggaagctgtgcggagacagaaactgctggaacagtccatccagagcgcccaggaaaccgagaagtccctgcacctgatccaggaaagcctgacattcatcgacaagcagctggccgcctatatcgccgacaaggtggacgccgcccagatgccacaggaagctcagaagatccagtccgacctgaccagccacgagatcagcctggaagagatgaagaagcacaaccagggcaaagaggccgcccagagggtcctgagccagatcgacgtggcccagaaaaaactgcaggacgtgtccatgaagttcaggctgttccagaagcccgccaacttcgagcagagactgcaggaatccaagatgatcctggatgaagtgaagatgcatctgccagccctggaaacaaagtccgtggaacaggaagtggtccagtcccagctgaaccactgcgtgaacctgtacaagagcctgtccgaagtgaagtccgaggtggaaatggtcatcaagaccggcagacagatcgtgcagaaaaagcagaccgagaaccccaaagaactggacgagagagtgaccgccctgaagctgcactacaacgagctgggcgccaaagtgacagagcggaaacagcagctggaaaagtgcctgaagctgtcccgcaagatgcggaaagaaatgaacgtgctgacagagtggctggctgccaccgacatggaactgaccaagagaagcgccgtggaaggcatgcccagcaacctggactccgaggtggcatggggcaaggccacccagaaagagatcgaaaagcagaaggtgcacctgaagtccatcaccgaagtgggcgaggctctgaaaaccgtgctgggcaagaaagaaaccctggtggaagataagctgagcctgctgaactctaactggatcgccgtgaccagcagagccgaggaatggctgaatctgctgctggaatatcagaaacacatggaaacctttgaccagaacgtggaccacatcaccaagtggatcatccaggctgacaccctgctggacgagtccgagaagaagaaacctcagcagaaagaagatgtgctgaagagactgaaggctgagctgaatgacatcagacccaaggtggacagcaccagggaccaggccgccaacctgatggccaaccacggcgaccactgcagaaaactggtggaaccccagatctccgagctgaatcacagattcgccgccatcagccacagaatcaagacaggcaaggccagcatccccctgaaagagctggaacagttcaacagcgacatccagaagctgctggaacccctggaagccgagatccagcagggcgtgaacctgaaagaagaggacttcaacaaggacatgaacgaggacaacgagggcacagtgaaagagctgctccagagaggcgacaacctgcagcagcgcatcaccgacgagagaaagcgcgaggaaatcaagatcaagcagcagctcctgcagaccaagcacaacgccctgaaggacctgagatcccagagaagaaagaaggccctggaaatcagccaccagtggtatcagtacaagagacaggccgacgacctgctgaaatgcctggacgacatcgagaagaagctggctagcctgcccgagcccagggacgagaggaagatcaaagaaatcgaccgggaactgcagaagaagaaagaggaactgaacgccgtccgcaggcaggccgagggcctgtctgaagatggcgccgctatggccgtggaacccacccagatccagctgagcaagagatggcgcgagatcgagagcaagttcgcccagttccgcagactgaacttcgcccagatccataccgtgcgggaagagacaatgatggtcatgacagaggacatgcccctggaaattagctacgtgcccagcacctacctgaccgagatcacacacgtgtcccaggcactgctggaagtggaacagctgctgaatgcccccgacctgtgcgccaaggacttcgaggatctgttcaagcaggaagagagcctgaagaatatcaaggactccctgcagcagtccagcggcagaatcgacatcatccacagcaagaaaacagccgccctgcagagcgctacccccgtggaacgcgtgaagctgcaggaagcactgagccagctggacttccagtgggagaaagtgaacaaaatgtacaaggaccggcagggcagattcgacagatccgtggaaaagtggcggagattccactacgacatcaagatcttcaatcagtggctgacagaggccgagcagttcctgagaaagacccagatccctgagaactgggagcacgccaagtacaagtggtatctgaaagaactgcaggatggcatcggccagagacagaccgtggtccgcacactgaacgccaccggcgaagagatcatccagcagagcagcaagaccgacgccagcatcctgcaggaaaagctgggctccctgaacctgagatggcaggaagtgtgcaagcagctgagcgacagaaagaaaaggctggaagaacagaagaatatcctgagcgagttccagagggacctgaacgagttcgtgctgtggctggaagaggctgacaatatcgcctccatccccctggaacccggcaaagagcagcagctgaaagaaaaactggaacaggtcaaactgctggtggaagaactgcctctgagacagggcagaatcctgaagcagctgaacgagacaggcggccctgtgctggtgtctgcccccatcagccccgaggaacaggacaaactggaaaacaaactgaagcagacaaacctgcagtggatcaaggtgtccagagccctgcccgagaagcagggggagatcgaggcccagatcaaggacctgggccagctggaaaaaaagctggaagatctggaagaacagctcaaccatctgctgctgtggctgagccccatcagaaaccagctggaaatctacaatcagcccaaccaggaaggccccttcgacgtcaaagaaaccgagatcgccgtgcaggctaagcagcctgacgtggaagagatcctgagcaagggacagcacctgtacaaagagaagcctgccacccagcccgtgaagcgcaaactggaagatctgtccagcgagtggaaggccgtgaaccgcctgctgcaggaactgagagccaagcagcccgacctggcccctggcctgacaacaatcggcgccagccccacccagacagtgaccctggtcacacagcccgtggtcacaaaagagacagccatcagcaagctggaaatgcccagctccctgatgctggaagtgcccgccctggccgacttcaacagagcctggaccgagctgaccgattggctgtctctgctggaccaggtcatcaagtcccagcgcgtgatggtcggcgatctggaagatatcaacgagatgatcatcaagcagaaagccaccatgcaggacctggaacagaggcggcctcagctggaagaactgatcacagccgcccagaacctgaaaaacaagaccagcaaccaggaagccaggaccatcatcaccgacagaatcgagaggatccagaatcagtgggacgaagtgcaggaacatctgcagaacagacgccagcagctgaatgagatgctgaaggacagcacccagtggctggaagctaaagaagaggctgaacaggtcctgggacaggccagagccaagctggaatcttggaaagagggcccctacaccgtcgacgctatccagaagaagatcaccgagacaaaacagctggccaaggacctgcggcagtggcagaccaacgtggacgtggccaacgacctggctctgaagctgctgcgggactacagcgccgacgacaccagaaaggtgcacatgatcacagagaacatcaacgcaagttggcggagcatccacaagagagtgtctgagcgcgaggctgcactggaagagactcacagactcctgcagcagttccccctggacctggaaaaattcctggcttggctgaccgaggctgagacaaccgccaacgtgctgcaggatgccaccagaaaagagagactgctggaagatagcaagggcgtgaaagaactgatgaagcagtggcaggacctgcagggcgaaatcgaggctcacaccgacgtgtaccacaacctggacgagaacagccagaagattctgagaagcctggaaggcagcgacgacgccgtgctgctgcagcggagactggacaacatgaacttcaagtggtccgagctgcgcaagaagtctctgaacatcagatcccatctggaagccagcagcgaccagtggaagagactgcacctgagtctgcaggaactgctggtctggctgcagctgaaggacgacgagctgagcagacaggcccccatcggcggcgatttccccgccgtgcagaaacagaacgacgtgcacagagccttcaagagagagctgaaaacaaaagaacccgtgatcatgagcaccctggaaactgtgcggatcttcctgaccgagcagcccctggaaggactggaaaagctgtaccaggaacccagagagctgccccctgaggaacgggcccagaacgtgacccggctgctgagaaagcaggccgaagaggtcaacaccgagtgggagaagctgaacctgcactccgccgactggcagagaaagatcgacgagacactggaacgcctgcaggaactgcaggaagctaccgacgagctggatctgaaactgcggcaggctgaagtgatcaagggcagctggcagcccgtgggggacctgctgatcgactctctgcaggaccatctggaaaaagtgaaggccctgaggggcgagatcgctcctctgaaagaaaacgtgtcccacgtgaacgacctggccaggcagctgaccaccctgggcatccagctgtccccctacaacctgagcactctggaagatctgaacaccagatggaagctgctgcaggtcgccgtggaagatagagtgcggcagctgcacgaagcccacagagacttcggccctgcctcccagcacttcctgtccacaagcgtgcagggcccctgggagagggccatcagccctaacaaggtgccctactacatcaaccacgagacacagaccacctgttgggaccaccccaagatgaccgagctgtatcagtctctggccgacctgaacaatgtgcggttcagcgcctacagaaccgctatgaagctgaggcgcctgcagaaagccctgtgcctggacctgctgagcctgagcgccgcctgtgacgccctggaccagcacaacctgaaacagaatgaccagcccatggatatcctgcagatcatcaactgcctgaccacaatctacgacaggctggaacaggaacacaacaacctggtcaacgtgcccctgtgcgtggacatgtgcctgaattggctgctgaacgtgtacgacaccggcagaaccggcaggatcagagtgctgtcctttaagaccggcatcatcagcctgtgcaaggcccacctggaagataagtaccgctatctgtttaaacaggtggccagctctaccggcttctgcgaccagagaaggctgggactgctgctgcacgactccatccagatccccagacagctgggagaggtggcctccttcggcggcagcaacatcgagcctagcgtgcggagctgcttccagttcgccaacaacaagcccgagatcgaagccgccctgttcctggattggatgaggctggaacctcagtctatggtctggctgcccgtgctgcacagggtggccgctgccgagacagccaagcaccaggccaagtgcaacatctgcaaagagtgccccatcatcggcttcagatatcggtccctgaagcacttcaactacgatatctgccagagctgcttcttcagcggcagagtggccaagggccacaagatgcattaccccatggtggaatactgcacccccaccaccagcggcgaggatgtgcgggacttcgccaaggtgctgaagaacaaattcaggactaagcgctacttcgctaagcaccctagaatgggctatctgcctgtgcagacagtgctggaaggcgacaacatggaaacccccgtgaccctgatcaacttttggcccgtggacagcgcacctgccagcagtcctcagctgagccacgacgacacccacagcagaatcgagcactacgcctccagactggccgagatggaaaacagcaacggcagctacctgaacgacagcatctcccccaacgagagcatcgacgacgagcatctgctgatccagcactactgccagtccctgaaccaggacagccccctgagccagcccagatcccctgcccagatcctgatctccctggaaagcgaggaaagaggcgagctggaaaggatcctggctgacctggaagaggaaaacagaaacctgcaggccgagtacgacagactgaagcagcagcacgagcacaagggcctgagccccctgcctagcccccctgagatgatgcccaccagccctcagagccccagggacgctgagctgatcgccgaggccaagctgctgaggcagcataagggccggctggaagcccggatgcagatcctggaagatcacaacaaacagctggaaagccagctgcacagactcagacagctgctggaacagccccaggccgaggctaaagtgaacggcaccacagtgtccagcccctccacctccctgcagagatccgacagcagccagcccatgctgctgagagtggtcggaagccagaccagcgacagcatgggcgaagaggatctgctgagcccccctcaggacaccagcacaggactggaagaagtgatggaacagctgaacaacagcttccccagcagcagaggcagaaacacccccggcaagcccatgcgcgaggacaccatgtga

SEQ ID NO: 2 - protein, 3686 aa, Homo sapiens
MLWWEEVEDCYEREDVQKKTFTKWVNAQFSKFGKQHIENLFSDLQDGRRLLDLLEGLTGQKLPKEKGSTRVHALNNVNKALRVLQNNNVDLVNIGSTDIVDGNHKLTLGLIWNIILHWQVKNVMKNIMAGLQQTNSEKILLSWVRQSTRNYPQVNVINFTTSWSDGLALNALIHSHRPDLFDWNSVVCQQSATQRLEHAFNIARYQLGIEKLLDPEDVDTTYPDKKSILMYITSLFQVLPQQVSIEAIQEVEMLPRPPKVTKEEHFQLHHQMHYSQQITVSLAQGYERTSSPKPRFKSYAYTQAAYVTTSDPTRSPFPSQHLEAPEDKSFGSSLMESEVNLDRYQTALEEVLSWLLSAEDTLQAQGEISNDVEVVKDQFHTHEGYMMDLTAHQGRVGNILQLGSKLIGTGKLSEDEETEVQEQMNLLNSRWECLRVASMEKQSNLHRVLMDLQNQKLKELNDWLTKTEERTRKMEEEPLGPDLEDLKRQVQQHKVLQEDLEQEQVRVNSLTHMVVVVDESSGDHATAALEEQLKVLGDRWANICRWTEDRWVLLQDILLKWQRLTEEQCLFSAWLSEKEDAVNKIHTTGFKDQNEMLSSLQKLAVLKADLEKKKQSMGKLYSLKQDLLSTLKNKSVTQKTEAWLDNFARCWDNLVQKLEKSTAQISQAVTTTQPSLTQTTVMETVTTVTTREQILVKHAQEELPPPPPQKKRQITVDSEIRKRLDVDITELHSWITRSEAVLQSPEFAIFRKEGNFSDLKEKVNAIEREKAEKFRKLQDASRSAQALVEQMVNEGVNADSIKQASEQLNSRWIEFCQLLSERLNWLEYQNNIIAFYNQLQQLEQMTTTAENWLKIQPTTPSEPTAIKSQLKICKDEVNRLSGLQPQIERLKIQSIALKEKGQGPMFLDADFVAFTNHFKQVFSDVQAREKELQTIFDTLPPMRYQETMSAIRTWVQQSETKLSIPQLSVTDYEIMEQRLGELQALQSSLQEQQSGLYYLSTTVKEMSKKAPSEISRKYQSEFEEIEGRWKKLSSQLVEHCQKLEEQMNKLRKIQNHIQTLKKWMAEVDVFLKEEWPALGDSEILKKQLKQCRLLVSDIQTIQPSLNSVNEGGQKIKNEAEPEFASRLETELKELNTQWDHMCQQVYARKEALKGGLEKTVSLQKDLSEMHEWMTQAEEEYLERDFEYKTPDELQKAVEEMKRAKEEAQQKEAKVKLLTESVNSVIAQAPPVAQEALKKELETLTTNYQWLCTRLNGKCKTLEEVWACWHELLSYLEKANKWLNEVEFKLKTTENIPGGAEEISEVLDSLENLMRHSEDNPNQIRILAQTLTDGGVMDELINEELETFNSRWRELHEEAVRRQKLLEQSIQSAQETEKSLHLIQESLTFIDKQLAAYIADKVDAAQMPQEAQKIQSDLTSHEISLEEMKKHNQGKEAAQRVLSQIDVAQKKLQDVSMKFRLFQKPANFEQRLQESKMILDEVKMHLPALETKSVEQEVVQSQLNHCVNLYKSLSEVKSEVEMVIKTGRQIVQKKQTENPKELDERVTALKLHYNELGAKVTERKQQLEKCLKLSRKMRKEMNVLTEWLAATDMELTKRSAVEGMPSNLDSEVAWGKATQKEIEKQKVHLKSITEVGEALKTVLGKKETLVEDKLSLLNSNWIAVTSRAEEWLNLLLEYQKHMETFDQNVDHITKWIIQADTLLDESEKKKPQQKEDVLKRLKAELNDIRPKVDSTRDQAANLMANHGDHCRKLVEPQISELNHRFAAISHRIKTGKASIPLKELEQFNSDIQKLLEPLEAEIQQGVNLKEEDFNKDMNEDNEGTVKELLQRGDNLQQRITDERKREEIKIKQQLLQTKHNALKDLRSQRRKKALEISHQWYQYKRQADDLLKCLDDIEKKLASLPEPRDERKIKEIDRELQKKKEELNAVRRQAEGLSEDGAAMAVEPTQIQLSKRWREIESKFAQFRRLNFAQIHTVREETMMVMTEDMPLEISYVPSTYLTEITHVSQALLEVEQLLNAPDLCAKDFEDLFKQEESLKNIKDSLQQSSGRIDIIHSKKTAALQSATPVERVKLQEALSQLDFQWEKVNKMYKDRQGRFDRSVEKWRRFHYDIKIFNQWLTEAEQFLRKTQIPENWEHAKYKWYLKELQDGIGQRQTVVRTLNATGEEIIQQSSKTDASILQEKLGSLNLRWQEVCKQLSDRKKRLEEQKNILSEFQRDLNEFVLWLEEADNIASIPLEPGKEQQLKEKLEQVKLLVEELPLRQGRILKQLNETGGPVLVSAPISPEEQDKLENKLKQTNLQWIKVSRALPEKQGEIEAQIKDLGQLEKKLEDLEEQLNHLLLWLSPIRNQLEIYNQPNQEGPFDVKETEIAVQAKQPDVEEILSKGQHLYKEKPATQPVKRKLEDLSSEWKAVNRLLQELRAKQPDLAPGLTTIGASPTQTVTLVTQPVVTKETAISKLEMPSSLMLEVPALADFNRAWTELTDWLSLLDQVIKSQRVMVGDLEDINEMIIKQKATMQDLEQRRPQLEELITAAQNLKNKTSNQEARTIITDRIERIQNQWDEVQEHLQNRRQQLNEMLKDSTQWLEAKEEAEQVLGQARAKLESWKEGPYTVDAIQKKITETKQLAKDLRQWQTNVDVANDLALKLLRDYSADDTRKVHMITENINASWRSIHKRVSEREAALEETHRLLQQFPLDLEKFLAWLTEAETTANVLQDATRKERLLEDSKGVKELMKQWQDLQGEIEAHTDVYHNLDENSQKILRSLEGSDDAVLLQRRLDNMNFKWSELRKKSLNIRSHLEASSDQWKRLHLSLQELLVWLQLKDDELSRQAPIGGDFPAVQKQNDVHRAFKRELKTKEPVIMSTLETVRIFLTEQPLEGLEKLYQEPRELPPEERAQNVTRLLRKQAEEVNTEWEKLNLHSADWQRKIDETLERLQELQEATDELDLKLRQAEVIKGSWQPVGDLLIDSLQDHLEKVKALRGEIAPLKENVSHVNDLARQLTTLGIQLSPYNLSTLEDLNTRWKLLQVAVEDRVRQLHEAHRDFGPASQHFLSTSVQGPWERAISPNKVPYYINHETQTTCWDHPKMTELYQSLADLNNVRFSAYRTAMKLRRLQKALCLDLLSLSAACDALDQHNLKQNDQPMDILQIINCLTTIYDRLEQEHNNLVNVPLCVDMCLNWLLNVYDTGRTGRIRVLSFKTGIISLCKAHLEDKYRYLFKQVASSTGFCDQRRLGLLLHDSIQIPRQLGEVASFGGSNIEPSVRSCFQFANNKPEIEAALFLDWMRLEPQSMVWLPVLHRVAAAETAKHQAKCNICKECPIIGFRYRSLKHFNYDICQSCFFSGRVAKGHKMHYPMVEYCTPTTSGEDVRDFAKVLKNKFRTKRYFAKHPRMGYLPVQTVLEGDNMETPVTLINFWPVDSAPASSPQLSHDDTHSRIEHYASRLAEMENSNGSYLNDSISPNESIDDEHLLIQHYCQSLNQDSPLSQPRSPAQILISLESEERGELERILADLEEENRNLQAEYDRLKQQHEHKGLSPLPSPPEMMPTSPQSPRDAELIAEAKLLRQHKGRLEARMQILEDHNKQLESQLHRLRQLLEQPQAEAKVNGTTVSSPSTSLQRSDSSQPMLLRVVGSQTSDSMGEEDLLSPPQDTSTGLEEVMEQLNNSFPSSRGRNTPGKPMREDTM

SEQ ID NO: 3 - DNA, 11067 bp, Artificial sequence
  Codon optimised dystrophin cDNA including Kozak sequence
gccaccatgctgtggtgggaggaagtggaagattgctacgagcgcgaggacgtgcagaagaaaaccttcaccaaatgggtcaacgcccagttcagcaagttcggcaagcagcacatcgagaacctgttcagcgacctgcaggacggcagaaggctgctggacctgctggaaggcctgaccggccagaagctgcccaaagagaagggcagcaccagagtgcacgccctgaacaacgtgaacaaggccctgagagtgctgcagaacaacaacgtggacctggtcaacatcggcagcaccgacatcgtggacggcaaccacaagctgaccctgggcctgatctggaacatcatcctgcactggcaggtcaaaaacgtgatgaagaacatcatggccggcctgcagcagaccaacagcgagaagatcctgctgagctgggtccgccagagcaccagaaactacccccaggtcaacgtgatcaacttcaccacctcttggagcgacggcctggccctgaacgccctgatccacagccacagacccgacctgttcgactggaacagcgtggtctgccagcagagcgccacccagagactggaacacgccttcaatatcgccagataccagctgggcatcgagaagctgctggatcccgaggacgtggacaccacctaccccgacaagaaatccatcctgatgtacatcaccagcctgttccaggtgctgccccagcaggtctccatcgaggccatccaggaagtggaaatgctgcccagaccccccaaagtgaccaaagaggaacacttccagctgcaccaccagatgcactacagccagcagatcaccgtgtccctggctcagggctacgagagaaccagcagccccaagcccagattcaagagctacgcctacacccaggccgcctacgtgaccaccagcgaccccaccagaagcccattccccagccagcacctggaagcccccgaggacaagagcttcggcagcagcctgatggaaagcgaagtgaacctggacagataccagaccgccctggaagaggtgctgtcctggctgctgtccgccgaggacacactgcaggcccagggcgagatcagcaacgacgtggaagtggtcaaagaccagttccacacccacgagggctacatgatggacctgaccgcccaccagggcagagtgggcaacatcctgcagctgggcagcaagctgatcggcaccggcaagctgagcgaggacgaagagacagaggtgcaggaacagatgaacctgctgaacagcagatgggagtgcctgagagtggccagcatggaaaagcagagcaacctgcacagagtgctgatggatctgcagaaccagaagctgaaagagctgaacgactggctgaccaagaccgaggaacggaccagaaagatggaagaggaacccctgggccccgacctggaagatctgaagagacaggtgcagcagcacaaggtgctgcaggaagatctggaacaggaacaggtccgcgtcaacagcctgacccacatggtggtggtggtggacgagagcagcggcgatcacgccaccgccgctctggaagaacagctgaaggtgctgggcgacagatgggccaacatctgccggtggaccgaggacagatgggtgctgctgcaggacatcctgctgaagtggcagagactgacagaggaacagtgcctgttctccgcctggctgagcgagaaagaggacgccgtcaacaagatccacaccaccggcttcaaggaccagaacgagatgctgagcagcctgcagaaactggccgtgctgaaggccgatctggaaaagaaaaagcagtccatgggcaagctgtacagcctgaagcaggacctgctgtccaccctgaagaacaagagcgtgacccagaaaaccgaggcctggctggacaacttcgccagatgctgggacaacctggtgcagaagctggaaaagagcaccgcccagatcagccaggccgtgaccacaacccagccctccctgacccagaccaccgtgatggaaaccgtgaccactgtgaccacccgcgagcagatcctggtcaaacacgcccaggaagaactgccccctccacccccccagaagaaaagacagatcacagtggacagcgagatcagaaagcggctggatgtggacatcaccgagctgcacagctggatcaccagatccgaggccgtgctgcagagccccgagttcgccatcttcagaaaagagggcaacttctccgacctgaaagaaaaagtgaacgccatcgagagagagaaggccgagaagttcagaaagctgcaggacgccagccgctctgctcaggctctggtggaacagatggtcaacgagggcgtgaacgccgacagcatcaagcaggccagcgagcagctgaactccagatggatcgagttctgccagctgctgtccgagagactgaactggctggaataccagaacaacatcattgccttctacaaccagctccagcagctggaacagatgaccaccaccgccgagaactggctgaagatccagcccaccacccccagcgagcccaccgccatcaagagccagctgaagatctgcaaggacgaagtgaacagactgtctggcctgcagccccagatcgagaggctgaagattcagtctatcgccctgaaagagaaaggccagggccccatgttcctggacgccgacttcgtggccttcaccaaccacttcaaacaggtgttctccgacgtgcaggccagagagaaagagctgcagaccatcttcgacaccctgccccccatgagataccaggaaaccatgagcgccatcagaacctgggtgcagcagagcgagacaaagctgagcatcccccagctgagcgtgaccgactacgagatcatggaacagagactgggcgagctgcaggctctgcagtccagtctgcaggaacagcagagcggcctgtactacctgagcaccaccgtgaaagagatgagcaagaaggccccctccgagatctccagaaagtaccagagcgagttcgaagagatcgagggcagatggaagaagctgtcctctcagctggtggaacactgccagaaactggaagaacagatgaacaagctgcggaagatccagaaccacatccagaccctgaaaaagtggatggccgaggtggacgtgttcctgaaagaggaatggcctgccctgggcgactccgagatcctgaaaaagcagctgaagcagtgcagactgctggtgtccgacatccagacaatccagcccagcctgaactccgtgaatgagggcggccagaagatcaagaacgaggccgagcctgagttcgccagcagactggaaaccgagctgaaagaactgaatacccagtgggaccacatgtgtcagcaggtctacgcccggaaagaggccctgaagggcggcctggaaaagaccgtgtctctgcagaaagacctgtccgagatgcacgagtggatgacccaggccgaggaagagtacctggaaagagacttcgagtacaagacccccgacgagctgcagaaagctgtggaagaaatgaagagggccaaagaagaggcccagcagaaagaggccaaagtcaagctgctgaccgagtccgtgaacagcgtgatcgcccaggcccctcccgtggctcaggaagccctgaagaaagaactggaaacactgaccaccaactaccagtggctgtgcaccagactgaacggcaagtgcaagaccctggaagaagtgtgggcctgctggcacgagctgctgagctacctggaaaaggccaacaagtggctgaacgaggtggaattcaagctgaaaaccaccgagaacatccctggcggcgctgaagagatcagcgaggtgctggacagcctggaaaacctgatgagacacagcgaggacaaccccaaccagatcagaatcctggcccagacactgaccgacggcggcgtgatggacgagctgatcaacgaggaactggaaaccttcaacagccggtggcgcgagctgcacgaggaagctgtgcggagacagaaactgctggaacagtccatccagagcgcccaggaaaccgagaagtccctgcacctgatccaggaaagcctgacattcatcgacaagcagctggccgcctatatcgccgacaaggtggacgccgcccagatgccacaggaagctcagaagatccagtccgacctgaccagccacgagatcagcctggaagagatgaagaagcacaaccagggcaaagaggccgcccagagggtcctgagccagatcgacgtggcccagaaaaaactgcaggacgtgtccatgaagttcaggctgttccagaagcccgccaacttcgagcagagactgcaggaatccaagatgatcctggatgaagtgaagatgcatctgccagccctggaaacaaagtccgtggaacaggaagtggtccagtcccagctgaaccactgcgtgaacctgtacaagagcctgtccgaagtgaagtccgaggtggaaatggtcatcaagaccggcagacagatcgtgcagaaaaagcagaccgagaaccccaaagaactggacgagagagtgaccgccctgaagctgcactacaacgagctgggcgccaaagtgacagagcggaaacagcagctggaaaagtgcctgaagctgtcccgcaagatgcggaaagaaatgaacgtgctgacagagtggctggctgccaccgacatggaactgaccaagagaagcgccgtggaaggcatgcccagcaacctggactccgaggtggcatggggcaaggccacccagaaagagatcgaaaagcagaaggtgcacctgaagtccatcaccgaagtgggcgaggctctgaaaaccgtgctgggcaagaaagaaaccctggtggaagataagctgagcctgctgaactctaactggatcgccgtgaccagcagagccgaggaatggctgaatctgctgctggaatatcagaaacacatggaaacctttgaccagaacgtggaccacatcaccaagtggatcatccaggctgacaccctgctggacgagtccgagaagaagaaacctcagcagaaagaagatgtgctgaagagactgaaggctgagctgaatgacatcagacccaaggtggacagcaccagggaccaggccgccaacctgatggccaaccacggcgaccactgcagaaaactggtggaaccccagatctccgagctgaatcacagattcgccgccatcagccacagaatcaagacaggcaaggccagcatccccctgaaagagctggaacagttcaacagcgacatccagaagctgctggaacccctggaagccgagatccagcagggcgtgaacctgaaagaagaggacttcaacaaggacatgaacgaggacaacgagggcacagtgaaagagctgctccagagaggcgacaacctgcagcagcgcatcaccgacgagagaaagcgcgaggaaatcaagatcaagcagcagctcctgcagaccaagcacaacgccctgaaggacctgagatcccagagaagaaagaaggccctggaaatcagccaccagtggtatcagtacaagagacaggccgacgacctgctgaaatgcctggacgacatcgagaagaagctggctagcctgcccgagcccagggacgagaggaagatcaaagaaatcgaccgggaactgcagaagaagaaagaggaactgaacgccgtccgcaggcaggccgagggcctgtctgaagatggcgccgctatggccgtggaacccacccagatccagctgagcaagagatggcgcgagatcgagagcaagttcgcccagttccgcagactgaacttcgcccagatccataccgtgcgggaagagacaatgatggtcatgacagaggacatgcccctggaaattagctacgtgcccagcacctacctgaccgagatcacacacgtgtcccaggcactgctggaagtggaacagctgctgaatgcccccgacctgtgcgccaaggacttcgaggatctgttcaagcaggaagagagcctgaagaatatcaaggactccctgcagcagtccagcggcagaatcgacatcatccacagcaagaaaacagccgccctgcagagcgctacccccgtggaacgcgtgaagctgcaggaagcactgagccagctggacttccagtgggagaaagtgaacaaaatgtacaaggaccggcagggcagattcgacagatccgtggaaaagtggcggagattccactacgacatcaagatcttcaatcagtggctgacagaggccgagcagttcctgagaaagacccagatccctgagaactgggagcacgccaagtacaagtggtatctgaaagaactgcaggatggcatcggccagagacagaccgtggtccgcacactgaacgccaccggcgaagagatcatccagcagagcagcaagaccgacgccagcatcctgcaggaaaagctgggctccctgaacctgagatggcaggaagtgtgcaagcagctgagcgacagaaagaaaaggctggaagaacagaagaatatcctgagcgagttccagagggacctgaacgagttcgtgctgtggctggaagaggctgacaatatcgcctccatccccctggaacccggcaaagagcagcagctgaaagaaaaactggaacaggtcaaactgctggtggaagaactgcctctgagacagggcagaatcctgaagcagctgaacgagacaggcggccctgtgctggtgtctgcccccatcagccccgaggaacaggacaaactggaaaacaaactgaagcagacaaacctgcagtggatcaaggtgtccagagccctgcccgagaagcagggggagatcgaggcccagatcaaggacctgggccagctggaaaaaaagctggaagatctggaagaacagctcaaccatctgctgctgtggctgagccccatcagaaaccagctggaaatctacaatcagcccaaccaggaaggccccttcgacgtcaaagaaaccgagatcgccgtgcaggctaagcagcctgacgtggaagagatcctgagcaagggacagcacctgtacaaagagaagcctgccacccagcccgtgaagcgcaaactggaagatctgtccagcgagtggaaggccgtgaaccgcctgctgcaggaactgagagccaagcagcccgacctggcccctggcctgacaacaatcggcgccagccccacccagacagtgaccctggtcacacagcccgtggtcacaaaagagacagccatcagcaagctggaaatgcccagctccctgatgctggaagtgcccgccctggccgacttcaacagagcctggaccgagctgaccgattggctgtctctgctggaccaggtcatcaagtcccagcgcgtgatggtcggcgatctggaagatatcaacgagatgatcatcaagcagaaagccaccatgcaggacctggaacagaggcggcctcagctggaagaactgatcacagccgcccagaacctgaaaaacaagaccagcaaccaggaagccaggaccatcatcaccgacagaatcgagaggatccagaatcagtgggacgaagtgcaggaacatctgcagaacagacgccagcagctgaatgagatgctgaaggacagcacccagtggctggaagctaaagaagaggctgaacaggtcctgggacaggccagagccaagctggaatcttggaaagagggcccctacaccgtcgacgctatccagaagaagatcaccgagacaaaacagctggccaaggacctgcggcagtggcagaccaacgtggacgtggccaacgacctggctctgaagctgctgcgggactacagcgccgacgacaccagaaaggtgcacatgatcacagagaacatcaacgcaagttggcggagcatccacaagagagtgtctgagcgcgaggctgcactggaagagactcacagactcctgcagcagttccccctggacctggaaaaattcctggcttggctgaccgaggctgagacaaccgccaacgtgctgcaggatgccaccagaaaagagagactgctggaagatagcaagggcgtgaaagaactgatgaagcagtggcaggacctgcagggcgaaatcgaggctcacaccgacgtgtaccacaacctggacgagaacagccagaagattctgagaagcctggaaggcagcgacgacgccgtgctgctgcagcggagactggacaacatgaacttcaagtggtccgagctgcgcaagaagtctctgaacatcagatcccatctggaagccagcagcgaccagtggaagagactgcacctgagtctgcaggaactgctggtctggctgcagctgaaggacgacgagctgagcagacaggcccccatcggcggcgatttccccgccgtgcagaaacagaacgacgtgcacagagccttcaagagagagctgaaaacaaaagaacccgtgatcatgagcaccctggaaactgtgcggatcttcctgaccgagcagcccctggaaggactggaaaagctgtaccaggaacccagagagctgccccctgaggaacgggcccagaacgtgacccggctgctgagaaagcaggccgaagaggtcaacaccgagtgggagaagctgaacctgcactccgccgactggcagagaaagatcgacgagacactggaacgcctgcaggaactgcaggaagctaccgacgagctggatctgaaactgcggcaggctgaagtgatcaagggcagctggcagcccgtgggggacctgctgatcgactctctgcaggaccatctggaaaaagtgaaggccctgaggggcgagatcgctcctctgaaagaaaacgtgtcccacgtgaacgacctggccaggcagctgaccaccctgggcatccagctgtccccctacaacctgagcactctggaagatctgaacaccagatggaagctgctgcaggtcgccgtggaagatagagtgcggcagctgcacgaagcccacagagacttcggccctgcctcccagcacttcctgtccacaagcgtgcagggcccctgggagagggccatcagccctaacaaggtgccctactacatcaaccacgagacacagaccacctgttgggaccaccccaagatgaccgagctgtatcagtctctggccgacctgaacaatgtgcggttcagcgcctacagaaccgctatgaagctgaggcgcctgcagaaagccctgtgcctggacctgctgagcctgagcgccgcctgtgacgccctggaccagcacaacctgaaacagaatgaccagcccatggatatcctgcagatcatcaactgcctgaccacaatctacgacaggctggaacaggaacacaacaacctggtcaacgtgcccctgtgcgtggacatgtgcctgaattggctgctgaacgtgtacgacaccggcagaaccggcaggatcagagtgctgtcctttaagaccggcatcatcagcctgtgcaaggcccacctggaagataagtaccgctatctgtttaaacaggtggccagctctaccggcttctgcgaccagagaaggctgggactgctgctgcacgactccatccagatccccagacagctgggagaggtggcctccttcggcggcagcaacatcgagcctagcgtgcggagctgcttccagttcgccaacaacaagcccgagatcgaagccgccctgttcctggattggatgaggctggaacctcagtctatggtctggctgcccgtgctgcacagggtggccgctgccgagacagccaagcaccaggccaagtgcaacatctgcaaagagtgccccatcatcggcttcagatatcggtccctgaagcacttcaactacgatatctgccagagctgcttcttcagcggcagagtggccaagggccacaagatgcattaccccatggtggaatactgcacccccaccaccagcggcgaggatgtgcgggacttcgccaaggtgctgaagaacaaattcaggactaagcgctacttcgctaagcaccctagaatgggctatctgcctgtgcagacagtgctggaaggcgacaacatggaaacccccgtgaccctgatcaacttttggcccgtggacagcgcacctgccagcagtcctcagctgagccacgacgacacccacagcagaatcgagcactacgcctccagactggccgagatggaaaacagcaacggcagctacctgaacgacagcatctcccccaacgagagcatcgacgacgagcatctgctgatccagcactactgccagtccctgaaccaggacagccccctgagccagcccagatcccctgcccagatcctgatctccctggaaagcgaggaaagaggcgagctggaaaggatcctggctgacctggaagaggaaaacagaaacctgcaggccgagtacgacagactgaagcagcagcacgagcacaagggcctgagccccctgcctagcccccctgagatgatgcccaccagccctcagagccccagggacgctgagctgatcgccgaggccaagctgctgaggcagcataagggccggctggaagcccggatgcagatcctggaagatcacaacaaacagctggaaagccagctgcacagactcagacagctgctggaacagccccaggccgaggctaaagtgaacggcaccacagtgtccagcccctccacctccctgcagagatccgacagcagccagcccatgctgctgagagtggtcggaagccagaccagcgacagcatgggcgaagaggatctgctgagcccccctcaggacaccagcacaggactggaagaagtgatggaacagctgaacaacagcttccccagcagcagaggcagaaacacccccggcaagcccatgcgcgaggacaccatgtga